European Patent Application EP 4 506 464 A1, published February 12, 2025. Title: CRISPR-Coacervate System. Applicant: ETH Zurich. Application EP. The sequence listing filed with the application follows.

SEQUENCE LISTING (47 sequences)

SEQ ID NO: 1 - RNA, 41 nt, synthetic construct
  source 1..41: mol_type = other RNA
taatttctactaagtgtagattgaagtagatatggcagcac

SEQ ID NO: 2 - RNA, 41 nt, synthetic construct
  source 1..41: mol_type = other RNA
taatttctactaagtgtagatacaatatgtgcttctacaca

SEQ ID NO: 3 - RNA, 150 nt, synthetic construct
  source 1..150: mol_type = other RNA
gaaggtggttagctacaggctgaccagtgcagttgtgtcatgtgctacggtgacctaacacgtcactcagtcacaacggctatctatatttccactaaccaaagttagtggaaatgtagatggttagcaccgaagaacgctgaagcgctg

SEQ ID NO: 4 - RNA, 53 nt, synthetic construct
  source 1..53: mol_type = other RNA
gaccaccccaaaaatgaaggggactaaaacatgcttctgtccagtgagcatgg

SEQ ID NO: 5 - RNA, 66 nt, synthetic construct
  source 1..66: mol_type = other RNA
tgactccctagaaccacgacagtttgccttgttgtagaagcttatcgtttggataggtatgacaac

SEQ ID NO: 6 - RNA, 63 nt, synthetic construct
  source 1..63: mol_type = other RNA
gttgatgagaagagcccaagatagagggcaataacactccctagaaccacgacagtttgcctt

SEQ ID NO: 7 - RNA, 180 nt, synthetic construct
  source 1..180: mol_type = other RNA
ttcactgataaagtggagaaccgcttcaccaaaagctgtcccttaggggattagaacttgagtgaaggtgggctgcttgcatcagcctaatgtcgagaagtgctttcttcggaaagtaaccctcgaaacaaattcatttgaaagaatgaaggaatgcaacacttgacacttaatgctcaa

SEQ ID NO: 8 - RNA, 182 nt, synthetic construct
  source 1..182: mol_type = other RNA
cttcactgataaagtggagaaccgcttcaccaaaagctgtcccttaggggattagaacttgagtgaaggtgggctgcttgcatcagcctaatgtcgagaagtgctttcttcggaaagtaaccctcgaaacaaattcatttggaatgcaacgaatgaaggaatgcaactcaactaatgtaact

SEQ ID NO: 9 - RNA, 46 nt, synthetic construct
  source 1..46: mol_type = other RNA
attgcgaccacacaatcgaagcgcagtaaggatggctagtgtaact

SEQ ID NO: 10-22 - skipped (13 entries)

SEQ ID NO: 23 - DNA, 10 bp, synthetic construct
  source 1..10: mol_type = other DNA
  misc_feature 1: note = labeled with FAM
  misc_feature 10: note = labeled with BHQ1
tttttttttt

SEQ ID NO: 24 - DNA, 11 bp, synthetic construct
  source 1..11: mol_type = other DNA
  misc_feature 1: note = labeled with FAM
  misc_feature 11: note = labeled with BHQ1
ttttttttttt

SEQ ID NO: 25 - DNA, 12 bp, synthetic construct
  source 1..12: mol_type = other DNA
  misc_feature 1: note = labeled with FAM
  misc_feature 12: note = labeled with BHQ1
tttttttttttt

SEQ ID NO: 26 - DNA, 15 bp, synthetic construct
  source 1..15: mol_type = other DNA
  misc_feature 1: note = labeled with FAM
  misc_feature 15: note = labeled with BHQ1
ttttttttttttttt

SEQ ID NO: 27-30 - skipped (4 entries)

SEQ ID NO: 31 - RNA, 15 nt, synthetic construct
  source 1..15: mol_type = other RNA
  misc_feature 1: note = labeled with FAM
  misc_feature 15: note = labeled with Biotin
aatggcaaaatggca

SEQ ID NO: 32-34 - skipped (3 entries)

SEQ ID NO: 35 - DNA, 24 bp, synthetic construct
  source 1..24: mol_type = other DNA
  misc_feature 1: note = labeled with FAM
  misc_feature 24: note = labeled with TAMRA
tagttgtgatgcwatcatgactag

SEQ ID NO: 36 - RNA, 45 nt, synthetic construct
  source 1..45: mol_type = other RNA
  misc_feature 1: note = labeled with cy5
  misc_feature 45: note = labeled with quencher
aaacgacggccagtgccaagcttactatacaacctactacctcat

SEQ ID NO: 37 - DNA, 18 bp, synthetic construct
  source 1..18: mol_type = other DNA
  misc_feature 1: note = labeled with (MethyleneBlue-Gold Nano Particles-Streptavidin) via a thiol group
  misc_feature 18: note = labeled with biotin
atgttgttctgcccatcg

SEQ ID NO: 38 - DNA, 10 bp, synthetic construct
  source 1..10: mol_type = other DNA
  misc_feature 1: note = carries an SH group
  misc_feature 10: note = labeled with Methylene Blue
ttttaatttt

SEQ ID NO: 39 - RNA, 20 nt, synthetic construct
  source 1..20: mol_type = other RNA
  misc_feature 1: note = carries an SH group connected via a C6 spacer
  misc_feature 20: note = labeled with Methylene Blue
tttttttttttttttttttt

SEQ ID NO: 40 - protein, 5 aa, synthetic construct
  REPEAT 1..5: note = the whole sequence is repeated from 2 to 600 times
  VAR_SEQ 4: note = X is any natural amino acid except proline
VPGXG

SEQ ID NO: 41 - protein, 8 aa, synthetic construct
  REPEAT 1..8: note = the whole sequence is repeated from 2 to 600 times
GRGDSPYS

SEQ ID NO: 42 - protein, 15 aa, synthetic construct
  REPEAT 1..15: note = the whole sequence is repeated from 2 to 600 times
GGRPSDSYGAPGGGN

SEQ ID NO: 43 - protein, 13 aa, synthetic construct
  REPEAT 1..13: note = the whole sequence is repated from 2 to 600 times
GYSGGRPGGQDLG

SEQ ID NO: 44 - protein, 11 aa, synthetic construct
  REPEAT 1..11: note = The whole sequence is repeated from 2 to 600 times
AQTPSSQYGAP

SEQ ID NO: 45 - skipped

SEQ ID NO: 46 - DNA, 12 bp, synthetic construct
  source 1..12: mol_type = other DNA
  misc_feature 1: note = labeled with FAM
  misc_feature 12: note = labeled with BHQ1
tttttttttttt

SEQ ID NO: 47 - skipped